European Patent Application EP 4 151 223 A1, published March 22, 2023. Title: Menopaussal symptoms improver. Applicant: KAO CORPORATION. The sequence listing filed with the application follows.

SEQUENCE LISTING (2 sequences)

SEQ ID NO: 1 - DNA, 27 bp, Artificial Sequence
  Synthetic oligonucleotide
caccatggcggattccagcgaaggccc

SEQ ID NO: 2 - DNA, 23 bp, Artificial Sequence
  Synthetic oligonucleotide
ctagagcggggcgtcatcagtcc